European Patent Specification EP 3 980 554 B1, published March 26, 2025. Title: Hybridizing all-LNA oligonucleotides. Applicant: F. Hoffmann-La Roche AG Roche Diagnostics GmbH. The sequence listing filed with the application follows.

SEQUENCE LISTING (70 sequences)

SEQ ID NO: 1 - DNA, 8 bp, Artificial Sequence
  Single-stranded oligonucleotide consisting of either D-LNA or L-LNA monomers; in the sequence of nucleobases a signifies adenine, t signifies thymine, u signifies uracil, g signifies guanine, and any c is either cytosine or 5-methylcytosine.
tgctcctg

SEQ ID NO: 2 - DNA, 8 bp, Artificial Sequence
  Single-stranded oligonucleotide consisting of either D-LNA or L-LNA monomers; in the sequence of nucleobases a signifies adenine, t signifies thymine, u signifies uracil, g signifies guanine, and any c is either cytosine or 5-methylcytosine.
caggagca

SEQ ID NO: 3 - DNA, 8 bp, Artificial Sequence
  Single-stranded oligonucleotide consisting of either D-LNA or L-LNA monomers; in the sequence of nucleobases a signifies adenine, t signifies thymine, u signifies uracil, g signifies guanine, and any c is either cytosine or 5-methylcytosine.
gcctgacg

SEQ ID NO: 4 - DNA, 8 bp, Artificial Sequence
  Single-stranded oligonucleotide consisting of either D-LNA or L-LNA monomers; in the sequence of nucleobases a signifies adenine, t signifies thymine, u signifies uracil, g signifies guanine, and any c is either cytosine or 5-methylcytosine.
cgtcaggc

SEQ ID NO: 5 - DNA, 10 bp, Artificial Sequence
  Single-stranded oligonucleotide consisting of either D-LNA or L-LNA monomers; in the sequence of nucleobases a signifies adenine, t signifies thymine, u signifies uracil, g signifies guanine, and any c is either cytosine or 5-methylcytosine.
ctgcctgacg

SEQ ID NO: 6 - DNA, 10 bp, Artificial Sequence
  Single-stranded oligonucleotide consisting of either D-LNA or L-LNA monomers; in the sequence of nucleobases a signifies adenine, t signifies thymine, u signifies uracil, g signifies guanine, and any c is either cytosine or 5-methylcytosine.
cgtcaggcag

SEQ ID NO: 7 - DNA, 12 bp, Artificial Sequence
  Single-stranded oligonucleotide consisting of either D-LNA or L-LNA monomers; in the sequence of nucleobases a signifies adenine, t signifies thymine, u signifies uracil, g signifies guanine, and any c is either cytosine or 5-methylcytosine.
gactgcctgacg

SEQ ID NO: 8 - DNA, 12 bp, Artificial Sequence
  Single-stranded oligonucleotide consisting of either D-LNA or L-LNA monomers; in the sequence of nucleobases a signifies adenine, t signifies thymine, u signifies uracil, g signifies guanine, and any c is either cytosine or 5-methylcytosine.
cgtcaggcagtc

SEQ ID NO: 9 - DNA, 9 bp, Artificial Sequence
  Single-stranded oligonucleotide consisting of either D-LNA or L-LNA monomers; in the sequence of nucleobases a signifies adenine, t signifies thymine, u signifies uracil, g signifies guanine, and any c is either cytosine or 5-methylcytosine.
tgctcctgt

SEQ ID NO: 10 - DNA, 9 bp, Artificial Sequence
  Single-stranded oligonucleotide consisting of either D-LNA or L-LNA monomers; in the sequence of nucleobases a signifies adenine, t signifies thymine, u signifies uracil, g signifies guanine, and any c is either cytosine or 5-methylcytosine.
acaggagca

SEQ ID NO: 11 - DNA, 8 bp, Artificial Sequence
  Single-stranded oligonucleotide consisting of either D-LNA or L-LNA monomers; in the sequence of nucleobases a signifies adenine, t signifies thymine, u signifies uracil, g signifies guanine, and any c is either cytosine or 5-methylcytosine.
gtgcgtct

SEQ ID NO: 12 - DNA, 8 bp, Artificial Sequence
  Single-stranded oligonucleotide consisting of either D-LNA or L-LNA monomers; in the sequence of nucleobases a signifies adenine, t signifies thymine, u signifies uracil, g signifies guanine, and any c is either cytosine or 5-methylcytosine.
agacgcac

SEQ ID NO: 13 - DNA, 8 bp, Artificial Sequence
  Single-stranded oligonucleotide consisting of either D-LNA or L-LNA monomers; in the sequence of nucleobases a signifies adenine, t signifies thymine, u signifies uracil, g signifies guanine, and any c is either cytosine or 5-methylcytosine.
gttggtgt

SEQ ID NO: 14 - DNA, 8 bp, Artificial Sequence
  Single-stranded oligonucleotide consisting of either D-LNA or L-LNA monomers; in the sequence of nucleobases a signifies adenine, t signifies thymine, u signifies uracil, g signifies guanine, and any c is either cytosine or 5-methylcytosine.
acaccaac

SEQ ID NO: 15 - DNA, 7 bp, Artificial Sequence
  Single-stranded oligonucleotide consisting of either D-LNA or L-LNA monomers; in the sequence of nucleobases a signifies adenine, t signifies thymine, u signifies uracil, g signifies guanine, and any c is either cytosine or 5-methylcytosine.
caggagc

SEQ ID NO: 16 - DNA, 6 bp, Artificial Sequence
  Single-stranded oligonucleotide consisting of either D-LNA or L-LNA monomers; in the sequence of nucleobases a signifies adenine, t signifies thymine, u signifies uracil, g signifies guanine, and any c is either cytosine or 5-methylcytosine.
gttggt

SEQ ID NO: 17 - DNA, 12 bp, Artificial Sequence
  Single-stranded oligonucleotide consisting of either D-LNA or L-LNA monomers; in the sequence of nucleobases a signifies adenine, t signifies thymine, u signifies uracil, g signifies guanine, and any c is either cytosine or 5-methylcytosine.
caacacaccaac

SEQ ID NO: 18 - DNA, 10 bp, Artificial Sequence
  Single-stranded oligonucleotide consisting of either D-LNA or L-LNA monomers; in the sequence of nucleobases a signifies adenine, t signifies thymine, u signifies uracil, g signifies guanine, and any c is either cytosine or 5-methylcytosine.
acacaccaac

SEQ ID NO: 19 - DNA, 7 bp, Artificial Sequence
  Single-stranded oligonucleotide consisting of either D-LNA or L-LNA monomers; in the sequence of nucleobases a signifies adenine, t signifies thymine, u signifies uracil, g signifies guanine, and any c is either cytosine or 5-methylcytosine.
caccaac

SEQ ID NO: 20 - DNA, 6 bp, Artificial Sequence
  Single-stranded oligonucleotide consisting of either D-LNA or L-LNA monomers; in the sequence of nucleobases a signifies adenine, t signifies thymine, u signifies uracil, g signifies guanine, and any c is either cytosine or 5-methylcytosine.
accaac

SEQ ID NO: 21 - DNA, 7 bp, Artificial Sequence
  Single-stranded oligonucleotide consisting of either D-LNA or L-LNA monomers; in the sequence of nucleobases a signifies adenine, t signifies thymine, u signifies uracil, g signifies guanine, and any c is either cytosine or 5-methylcytosine.
gttggtg

SEQ ID NO: 22 - DNA, 9 bp, Artificial Sequence
  Single-stranded oligonucleotide consisting of either D-LNA or L-LNA monomers; in the sequence of nucleobases a signifies adenine, t signifies thymine, u signifies uracil, g signifies guanine, and any c is either cytosine or 5-methylcytosine.
gttggtgtg

SEQ ID NO: 23 - DNA, 12 bp, Artificial Sequence
  Single-stranded oligonucleotide consisting of either D-LNA or L-LNA monomers; in the sequence of nucleobases a signifies adenine, t signifies thymine, u signifies uracil, g signifies guanine, and any c is either cytosine or 5-methylcytosine.
gttggtgtgttg

SEQ ID NO: 24 - DNA, 9 bp, Artificial Sequence
  Single-stranded oligonucleotide consisting of either D-LNA or L-LNA monomers; in the sequence of nucleobases a signifies adenine, t signifies thymine, u signifies uracil, g signifies guanine, and any c is either cytosine or 5-methylcytosine.
ttttttttt

SEQ ID NO: 25 - DNA, 8 bp, Artificial Sequence
  Single-stranded oligonucleotide consisting of either D-LNA or L-LNA monomers; in the sequence of nucleobases a signifies adenine, t signifies thymine, u signifies uracil, g signifies guanine, and any c is either cytosine or 5-methylcytosine.
tttttttt

SEQ ID NO: 26 - DNA, 7 bp, Artificial Sequence
  Single-stranded oligonucleotide consisting of either D-LNA or L-LNA monomers; in the sequence of nucleobases a signifies adenine, t signifies thymine, u signifies uracil, g signifies guanine, and any c is either cytosine or 5-methylcytosine.
ttttttt

SEQ ID NO: 27 - DNA, 6 bp, Artificial Sequence
  Single-stranded oligonucleotide consisting of either D-LNA or L-LNA monomers; in the sequence of nucleobases a signifies adenine, t signifies thymine, u signifies uracil, g signifies guanine, and any c is either cytosine or 5-methylcytosine.
tttttt

SEQ ID NO: 28 - DNA, 9 bp, Artificial Sequence
  Single-stranded oligonucleotide consisting of either D-LNA or L-LNA monomers; in the sequence of nucleobases a signifies adenine, t signifies thymine, u signifies uracil, g signifies guanine, and any c is either cytosine or 5-methylcytosine.
aaaaaaaaa

SEQ ID NO: 29 - DNA, 4 bp, Artificial Sequence
  Single-stranded oligonucleotide consisting of either D-LNA or L-LNA monomers; in the sequence of nucleobases a signifies adenine, t signifies thymine, u signifies uracil, g signifies guanine, and any c is either cytosine or 5-methylcytosine.
tttt

SEQ ID NO: 30 - DNA, 9 bp, Artificial Sequence
  Single-stranded oligonucleotide consisting of either D-LNA or L-LNA monomers; in the sequence of nucleobases a signifies adenine, t signifies thymine, u signifies uracil, g signifies guanine, and any c is either cytosine or 5-methylcytosine.
cacaccaac

SEQ ID NO: 31 - DNA, 15 bp, Artificial Sequence
  Single-stranded oligonucleotide consisting of either D-LNA or L-LNA monomers; in the sequence of nucleobases a signifies adenine, t signifies thymine, u signifies uracil, g signifies guanine, and any c is either cytosine or 5-methylcytosine.
gttggtgtgttggtg

SEQ ID NO: 32 - DNA, 15 bp, Artificial Sequence
  Single-stranded oligonucleotide consisting of either D-LNA or L-LNA monomers; in the sequence of nucleobases a signifies adenine, t signifies thymine, u signifies uracil, g signifies guanine, and any c is either cytosine or 5-methylcytosine.
caccaacacaccaac

SEQ ID NO: 33 - DNA, 5 bp, Artificial Sequence
  Single-stranded oligonucleotide consisting of either D-LNA or L-LNA monomers; in the sequence of nucleobases a signifies adenine, t signifies thymine, u signifies uracil, g signifies guanine, and any c is either cytosine or 5-methylcytosine.
cttcc

SEQ ID NO: 34 - DNA, 5 bp, Artificial Sequence
  Single-stranded oligonucleotide consisting of either D-LNA or L-LNA monomers; in the sequence of nucleobases a signifies adenine, t signifies thymine, u signifies uracil, g signifies guanine, and any c is either cytosine or 5-methylcytosine.
ggaag

SEQ ID NO: 35 - DNA, 6 bp, Artificial Sequence
  Single-stranded oligonucleotide consisting of either D-LNA or L-LNA monomers; in the sequence of nucleobases a signifies adenine, t signifies thymine, u signifies uracil, g signifies guanine, and any c is either cytosine or 5-methylcytosine.
tcttcc

SEQ ID NO: 36 - DNA, 6 bp, Artificial Sequence
  Single-stranded oligonucleotide consisting of either D-LNA or L-LNA monomers; in the sequence of nucleobases a signifies adenine, t signifies thymine, u signifies uracil, g signifies guanine, and any c is either cytosine or 5-methylcytosine.
ggaaga

SEQ ID NO: 37 - DNA, 9 bp, Artificial Sequence
  Single-stranded oligonucleotide consisting of either D-LNA or L-LNA monomers; in the sequence of nucleobases a signifies adenine, t signifies thymine, u signifies uracil, g signifies guanine, and any c is either cytosine or 5-methylcytosine.
ttctcttcc

SEQ ID NO: 38 - DNA, 9 bp, Artificial Sequence
  Single-stranded oligonucleotide consisting of either D-LNA or L-LNA monomers; in the sequence of nucleobases a signifies adenine, t signifies thymine, u signifies uracil, g signifies guanine, and any c is either cytosine or 5-methylcytosine.
ggaagagaa

SEQ ID NO: 39 - DNA, 6 bp, Artificial Sequence
  Single-stranded oligonucleotide consisting of either D-LNA or L-LNA monomers; in the sequence of nucleobases a signifies adenine, t signifies thymine, u signifies uracil, g signifies guanine, and any c is either cytosine or 5-methylcytosine.
aaaaaa

SEQ ID NO: 40 - DNA, 6 bp, Artificial Sequence
  Single-stranded oligonucleotide consisting of either D-LNA or L-LNA monomers; in the sequence of nucleobases a signifies adenine, t signifies thymine, u signifies uracil, g signifies guanine, and any c is either cytosine or 5-methylcytosine.
ctgtca

SEQ ID NO: 41 - DNA, 6 bp, Artificial Sequence
  Single-stranded oligonucleotide consisting of either D-LNA or L-LNA monomers; in the sequence of nucleobases a signifies adenine, t signifies thymine, u signifies uracil, g signifies guanine, and any c is either cytosine or 5-methylcytosine.
tgacag

SEQ ID NO: 42 - DNA, 5 bp, Artificial Sequence
  Single-stranded oligonucleotide consisting of either D-LNA or L-LNA monomers; in the sequence of nucleobases a signifies adenine, t signifies thymine, u signifies uracil, g signifies guanine, and any c is either cytosine or 5-methylcytosine.
gctcc

SEQ ID NO: 43 - DNA, 5 bp, Artificial Sequence
  Single-stranded oligonucleotide consisting of either D-LNA or L-LNA monomers; in the sequence of nucleobases a signifies adenine, t signifies thymine, u signifies uracil, g signifies guanine, and any c is either cytosine or 5-methylcytosine.
ggagc

SEQ ID NO: 44 - DNA, 6 bp, Artificial Sequence
  Single-stranded oligonucleotide consisting of either D-LNA or L-LNA monomers; in the sequence of nucleobases a signifies adenine, t signifies thymine, u signifies uracil, g signifies guanine, and any c is either cytosine or 5-methylcytosine.
tgctcc

SEQ ID NO: 45 - DNA, 6 bp, Artificial Sequence
  Single-stranded oligonucleotide consisting of either D-LNA or L-LNA monomers; in the sequence of nucleobases a signifies adenine, t signifies thymine, u signifies uracil, g signifies guanine, and any c is either cytosine or 5-methylcytosine.
ggagca

SEQ ID NO: 46 - DNA, 5 bp, Artificial Sequence
  Single-stranded oligonucleotide consisting of either D-LNA or L-LNA monomers; in the sequence of nucleobases a signifies adenine, t signifies thymine, u signifies uracil, g signifies guanine, and any c is either cytosine or 5-methylcytosine.
ccaac

SEQ ID NO: 47 - DNA, 15 bp, Artificial Sequence
  Single-stranded oligonucleotide consisting of either D-LNA or L-LNA monomers; in the sequence of nucleobases a signifies adenine, t signifies thymine, u signifies uracil, g signifies guanine, and any c is either cytosine or 5-methylcytosine.
cgtcaggcagttcag

SEQ ID NO: 48 - DNA, 15 bp, Artificial Sequence
  Single-stranded oligonucleotide consisting of either D-LNA or L-LNA monomers; in the sequence of nucleobases a signifies adenine, t signifies thymine, u signifies uracil, g signifies guanine, and any c is either cytosine or 5-methylcytosine.
ctgaactgcctgacg

SEQ ID NO: 49 - DNA, 4 bp, Artificial Sequence
  Single-stranded oligonucleotide consisting of either D-LNA or L-LNA monomers; in the sequence of nucleobases a signifies adenine, t signifies thymine, u signifies uracil, g signifies guanine, and any c is either cytosine or 5-methylcytosine.
tttt

SEQ ID NO: 50 - DNA, 15 bp, Artificial Sequence
  Single-stranded oligonucleotide consisting of either D-LNA or L-LNA monomers; in the sequence of nucleobases a signifies adenine, t signifies thymine, u signifies uracil, g signifies guanine, and any c is either cytosine or 5-methylcytosine.
gttggtgtgttggtg

SEQ ID NO: 51 - DNA, 5 bp, Artificial Sequence
  Single-stranded oligonucleotide consisting of either D-LNA or L-LNA monomers; in the sequence of nucleobases a signifies adenine, t signifies thymine, u signifies uracil, g signifies guanine, and any c is either cytosine or 5-methylcytosine.
cttcc

SEQ ID NO: 52 - DNA, 12 bp, Artificial Sequence
  Single-stranded oligonucleotide consisting of either D-LNA or L-LNA monomers; in the sequence of nucleobases a signifies adenine, t signifies thymine, u signifies uracil, g signifies guanine, and any c is either cytosine or 5-methylcytosine.
caacacaccaac

SEQ ID NO: 53 - DNA, 12 bp, Artificial Sequence
  Single-stranded oligonucleotide consisting of either D-LNA or L-LNA monomers; in the sequence of nucleobases a signifies adenine, t signifies thymine, u signifies uracil, g signifies guanine, and any c is either cytosine or 5-methylcytosine.
gttggtgtgttg

SEQ ID NO: 54 - DNA, 15 bp, Artificial Sequence
  Single-stranded oligonucleotide consisting of either D-LNA or L-LNA monomers; in the sequence of nucleobases a signifies adenine, t signifies thymine, u signifies uracil, g signifies guanine, and any c is either cytosine or 5-methylcytosine.
caccaacacaccaac

SEQ ID NO: 55 - DNA, 15 bp, Artificial Sequence
  Single-stranded oligonucleotide consisting of either D-LNA or L-LNA monomers; in the sequence of nucleobases a signifies adenine, t signifies thymine, u signifies uracil, g signifies guanine, and any c is either cytosine or 5-methylcytosine.
cgtcaggcagttcag

SEQ ID NO: 56 - DNA, 4 bp, Artificial Sequence
  Single-stranded oligonucleotide consisting of either D-LNA or L-LNA monomers; in the sequence of nucleobases a signifies adenine, t signifies thymine, u signifies uracil, g signifies guanine, and any c is either cytosine or 5-methylcytosine.
caac

SEQ ID NO: 57 - DNA, 5 bp, Artificial Sequence
  Single-stranded oligonucleotide consisting of either D-LNA or L-LNA monomers; in the sequence of nucleobases a signifies adenine, t signifies thymine, u signifies uracil, g signifies guanine, and any c is either cytosine or 5-methylcytosine.
ttttt

SEQ ID NO: 58 - DNA, 4 bp, Artificial Sequence
  Single-stranded oligonucleotide consisting of either D-LNA or L-LNA monomers; in the sequence of nucleobases a signifies adenine, t signifies thymine, u signifies uracil, g signifies guanine, and any c is either cytosine or 5-methylcytosine.
tttt

SEQ ID NO: 59 - DNA, 20 bp, Artificial Sequence
  Single-stranded oligonucleotide consisting of either D-LNA or L-LNA monomers; in the sequence of nucleobases a signifies adenine, t signifies thymine, u signifies uracil, g signifies guanine, and any c is either cytosine or 5-methylcytosine.
cagtggacgacgatagacat

SEQ ID NO: 60 - DNA, 20 bp, Artificial Sequence
  Single-stranded oligonucleotide consisting of either D-LNA or L-LNA monomers; in the sequence of nucleobases a signifies adenine, t signifies thymine, u signifies uracil, g signifies guanine, and any c is either cytosine or 5-methylcytosine.
atgtctatcgtcgtccactg

SEQ ID NO: 61 - DNA, 20 bp, Artificial Sequence
  Single-stranded oligonucleotide consisting of either D-LNA or L-LNA monomers; in the sequence of nucleobases a signifies adenine, t signifies thymine, u signifies uracil, g signifies guanine, and any c is either cytosine or 5-methylcytosine.
agaggatcgaggagtacagg

SEQ ID NO: 62 - DNA, 20 bp, Artificial Sequence
  Single-stranded oligonucleotide consisting of either D-LNA or L-LNA monomers; in the sequence of nucleobases a signifies adenine, t signifies thymine, u signifies uracil, g signifies guanine, and any c is either cytosine or 5-methylcytosine.
cctgtactcctcgatcctct

SEQ ID NO: 63 - DNA, 20 bp, Artificial Sequence
  Single-stranded oligonucleotide consisting of either D-LNA or L-LNA monomers; in the sequence of nucleobases a signifies adenine, t signifies thymine, u signifies uracil, g signifies guanine, and any c is either cytosine or 5-methylcytosine.
agaaatggacgagatgctaa

SEQ ID NO: 64 - DNA, 20 bp, Artificial Sequence
  Single-stranded oligonucleotide consisting of either D-LNA or L-LNA monomers; in the sequence of nucleobases a signifies adenine, t signifies thymine, u signifies uracil, g signifies guanine, and any c is either cytosine or 5-methylcytosine.
ttagcatctcgtccatttct

SEQ ID NO: 65 - DNA, 20 bp, Artificial Sequence
  Single-stranded oligonucleotide consisting of either D-LNA or L-LNA monomers; in the sequence of nucleobases a signifies adenine, t signifies thymine, u signifies uracil, g signifies guanine, and any c is either cytosine or 5-methylcytosine.
actgaacttgtgagaaacgc

SEQ ID NO: 66 - DNA, 20 bp, Artificial Sequence
  Single-stranded oligonucleotide consisting of either D-LNA or L-LNA monomers; in the sequence of nucleobases a signifies adenine, t signifies thymine, u signifies uracil, g signifies guanine, and any c is either cytosine or 5-methylcytosine.
gcgtttctcacaagttcagt

SEQ ID NO: 67 - DNA, 20 bp, Artificial Sequence
  Single-stranded oligonucleotide consisting of either D-LNA or L-LNA monomers; in the sequence of nucleobases a signifies adenine, t signifies thymine, u signifies uracil, g signifies guanine, and any c is either cytosine or 5-methylcytosine.
atggagagtcaggcaagttt

SEQ ID NO: 68 - DNA, 20 bp, Artificial Sequence
  Single-stranded oligonucleotide consisting of either D-LNA or L-LNA monomers; in the sequence of nucleobases a signifies adenine, t signifies thymine, u signifies uracil, g signifies guanine, and any c is either cytosine or 5-methylcytosine.
aaacttgcctgactctccat

SEQ ID NO: 69 - DNA, 20 bp, Artificial Sequence
  Single-stranded oligonucleotide consisting of either D-LNA or L-LNA monomers; in the sequence of nucleobases a signifies adenine, t signifies thymine, u signifies uracil, g signifies guanine, and any c is either cytosine or 5-methylcytosine.
tgaagatgcgagtgatgaac

SEQ ID NO: 70 - DNA, 20 bp, Artificial Sequence
  Single-stranded oligonucleotide consisting of either D-LNA or L-LNA monomers; in the sequence of nucleobases a signifies adenine, t signifies thymine, u signifies uracil, g signifies guanine, and any c is either cytosine or 5-methylcytosine.
gttcatcactcgcatcttca